European Patent Application EP 4 582 543 A1, published July 9, 2025. Title: 基因PRDX5和GPX4在制备去势抵抗性前列腺癌的药物中的应用. Applicant: 江南大学. Application WO. The sequence listing filed with the application follows.

SEQUENCE LISTING (14 sequences)

SEQ ID NO: 1 - RNA, 21 nt, synthetic construct
  source 1..21: mol_type = other RNA
cagacttattactagatgatt

SEQ ID NO: 2 - RNA, 23 nt, synthetic construct
  source 1..23: mol_type = other RNA
aatcatctagtaataagtctgtc

SEQ ID NO: 3 - RNA, 21 nt, synthetic construct
  source 1..21: mol_type = other RNA
acaacgtcaaattcgatatgt

SEQ ID NO: 4 - RNA, 23 nt, synthetic construct
  source 1..23: mol_type = other RNA
acatatcgaatttgacgttgtac

SEQ ID NO: 5 - RNA, 21 nt, synthetic construct
  source 1..21: mol_type = other RNA
gtgaggcaagaccgaagtaaa

SEQ ID NO: 6 - RNA, 23 nt, synthetic construct
  source 1..23: mol_type = other RNA
tttacttcggtcttgcctcactg

SEQ ID NO: 7 - RNA, 25 nt, synthetic construct
  source 1..25: mol_type = other RNA
agacagacttattactagatgattc

SEQ ID NO: 8 - RNA, 27 nt, synthetic construct
  source 1..27: mol_type = other RNA
gaatcatctagtaataagtctgtctcc

SEQ ID NO: 9 - RNA, 25 nt, synthetic construct
  source 1..25: mol_type = other RNA
ggccagatttctgcaataaacactt

SEQ ID NO: 10 - RNA, 27 nt, synthetic construct
  source 1..27: mol_type = other RNA
aagtgtttattgcagaaatctggccaa

SEQ ID NO: 11 - RNA, 25 nt, synthetic construct
  source 1..25: mol_type = other RNA
gtgaggcaagaccgaagtaaactac

SEQ ID NO: 12 - RNA, 27 nt, synthetic construct
  source 1..27: mol_type = other RNA
gtagtttacttcggtcttgcctcactg

SEQ ID NO: 13 - RNA, 25 nt, synthetic construct
  source 1..25: mol_type = other RNA
ctacaacgtcaaattcgatatgttc

SEQ ID NO: 14 - RNA, 27 nt, synthetic construct
  source 1..27: mol_type = other RNA
gaacatatcgaatttgacgttgtagcc